European Patent Application EP 4 378 480 A1, published June 5, 2024. Title: Anti-hapetitis B virus agent targeting host factor LIPG. Applicant: ピューロテックバイオ株式会社. Application JP. The sequence listing filed with the application follows.

SEQUENCE LISTING (138 sequences)

SEQ ID NO: 1 - protein, 16 aa, synthetic construct
  REGION 1..16: note = LIPH4-23
LNCRDNTRPVMSAMTC

SEQ ID NO: 2 - protein, 16 aa, synthetic construct
  REGION 1..16: note = LIPH4-44
SCSFAVLSDTQPQAHS

SEQ ID NO: 3 - protein, 16 aa, synthetic construct
  REGION 1..16: note = LIPH4-73
DAFAATARDEYRAARN

SEQ ID NO: 4 - protein, 16 aa, synthetic construct
  REGION 1..16: note = LIPH4-90
LCECRDVLSCYYITDT

SEQ ID NO: 5 - protein, 16 aa, synthetic construct
  REGION 1..16: note = LIPH4-42
LGPGVETCSWQCCSDL

SEQ ID NO: 6 - protein, 16 aa, synthetic construct
  REGION 1..16: note = LIPH4-17
CMLDRLACFGEILLVQ

SEQ ID NO: 7 - protein, 16 aa, synthetic construct
  REGION 1..16: note = LIPH4-4
PRYHWNSTSMFNSESP

SEQ ID NO: 8 - protein, 16 aa, synthetic construct
  REGION 1..16: note = LIPH4-16
CPCVNGATRHRPTSLC

SEQ ID NO: 9 - protein, 9 aa, synthetic construct
  REGION 1..9: note = LIPH4-74
IRNVNHSDH

SEQ ID NO: 10 - protein, 9 aa, synthetic construct
  REGION 1..9: note = LIPH4-81
NSSDARGCD

SEQ ID NO: 11 - protein, 9 aa, synthetic construct
  REGION 1..9: note = LIPH4-87
GADLRRGCC

SEQ ID NO: 12 - protein, 9 aa, synthetic construct
  REGION 1..9: note = LIPH4-94
AMHIDRRFR

SEQ ID NO: 13 - protein, 9 aa, synthetic construct
  REGION 1..9: note = LIPH4-64
DLSFSAPNF

SEQ ID NO: 14 - protein, 9 aa, synthetic construct
  REGION 1..9: note = LIPH4-14
RCRQSWNTM

SEQ ID NO: 15 - protein, 9 aa, synthetic construct
  REGION 1..9: note = LIPH4-2
SLYTGFRAH

SEQ ID NO: 16 - protein, 9 aa, synthetic construct
  REGION 1..9: note = LIPH4-8
MRKVSVKTS

SEQ ID NO: 17 - protein, 9 aa, synthetic construct
  REGION 1..9: note = LIPH4-12
LVPWLRYAY

SEQ ID NO: 18 - protein, 9 aa, synthetic construct
  REGION 1..9: note = LIPH4-15
LNVGYVFYP

SEQ ID NO: 19 - protein, 9 aa, synthetic construct
  REGION 1..9: note = LIPH4-70
PPAQRSYIQ

SEQ ID NO: 20 - protein, 9 aa, synthetic construct
  REGION 1..9: note = LIPH4-71
SRSPPGRRM

SEQ ID NO: 21 - protein, 16 aa, synthetic construct
  REGION 1..16: note = LIPH4-NTNA
RKSGGVCLNCRHNTAG

SEQ ID NO: 22 - protein, 16 aa, synthetic construct
  REGION 1..16: note = LIPH4-NTNB
LNCRHNTAGRHCHYCK

SEQ ID NO: 23 - protein, 8 aa, synthetic construct
  REGION 1..8: note = LIPH4-23s
LNCRDNTR

SEQ ID NO: 24 - protein, 8 aa, synthetic construct
  REGION 1..8: note = LIPH4-23SA
LNARDNTR

SEQ ID NO: 25 - protein, 8 aa, synthetic construct
  REGION 1..8: note = LIPH4-NTNBs
NCRHNTAG

SEQ ID NO: 26 - protein, 8 aa, synthetic construct
  REGION 1..8: note = LIPH4-NTNBsA
NARHNTAG

SEQ ID NO: 27 - DNA, 1815 bp, Homo sapiens
  source 1..1815: mol_type = other DNA
  CDS 1..1815
atgatgcgcgcagtgtgggaggcgctggcggcgctggcggcggtggcgtgcctggtgggcgcggtgcgcggcgggcccgggctcagcatgttcgcgggccaggcggcgcagcccgatccctgctcggacgagaacggccacccgcgccgctgcatcccggactttgtcaatgcggccttcggcaaggacgtgcgcgtgtccagcacctgcggccggcccccggcgcgctactgcgtggtgagcgagcgcggcgaggagcggctgcgctcgtgccacctctgcaacgcgtccgaccccaagaaggcgcacccgcccgccttcctcaccgacctcaacaacccgcacaacctgacgtgctggcagtccgagaactacctgcagttcccgcacaacgtcacgctcacactgtccctcggcaagaagttcgaagtgacctacgtgagcctgcagttctgctcgccgcggcccgagtccatggccatctacaagtccatggactacgggcgcacgtgggtgcccttccagttctactccacgcagtgccgcaagatgtacaaccggccgcaccgcgcgcccatcaccaagcagaacgagcaggaggccgtgtgcaccgactcgcacaccgacatgcgcccgctctcgggcggcctcatcgccttcagcacgctggacgggcggccctcggcgcacgacttcgacaactcgcccgtgctgcaggactgggtcacggccacagacatccgcgtggccttcagccgcctgcacacgttcggcgacgagaacgaggacgactcggagctggcgcgcgactcgtacttctacgcggtgtccgacctgcaggtgggcggccggtgcaagtgcaacggccacgcggcccgctgcgtgcgcgaccgcgacgacagcctggtgtgcgactgcaggcacaacacggccggcccggagtgcgaccgctgcaagcccttccactacgaccggccctggcagcgcgccacagcccgcgaagccaacgagtgcgtggcctgtaactgcaacctgcatgcccggcgctgccgcttcaacatggagctctacaagctttcggggcgcaagagcggaggtgtctgcctcaactgtcgccacaacaccgccggccgccactgccattactgcaaggagggctactaccgcgacatgggcaagcccatcacccaccggaaggcctgcaaagcctgtgattgccaccctgtgggtgctgctggcaaaacctgcaaccaaaccaccggccagtgtccctgcaaggacggcgtgacgggtatcacctgcaaccgctgcgccaaaggctaccagcagagccgctctcccatcgccccctgcataaagatccctgtagcgccgccgacgactgcagccagcagcgtggaggagcctgaagactgcgattcctactgcaaggcctccaaggggaagctgaagattaacatgaaaaagtactgcaagaaggactatgccgtccagatccacatcctgaaggcggacaaggcgggggactggtggaagttcacggtgaacatcatctccgtgtataagcagggcacgagccgcatccgccgcggtgaccagagcctgtggatccgctcgcgggacatcgcctgcaagtgtcccaaaatcaagcccctcaagaagtacctgctgctgggcaacgcggaggactctccggaccagagcggcatcgtggccgataaaagcagcctggtgatccagtggcgggacacgtgggcgcggcggctgcgcaagttccagcagcgtgagaagaagggcaagtgcaagaaggcctag

SEQ ID NO: 28 - protein, 604 aa, Homo sapiens
MMRAVWEALAALAAVACLVGAVRGGPGLSMFAGQAAQPDPCSDENGHPRRCIPDFVNAAFGKDVRVSSTCGRPPARYCVVSERGEERLRSCHLCNASDPKKAHPPAFLTDLNNPHNLTCWQSENYLQFPHNVTLTLSLGKKFEVTYVSLQFCSPRPESMAIYKSMDYGRTWVPFQFYSTQCRKMYNRPHRAPITKQNEQEAVCTDSHTDMRPLSGGLIAFSTLDGRPSAHDFDNSPVLQDWVTATDIRVAFSRLHTFGDENEDDSELARDSYFYAVSDLQVGGRCKCNGHAARCVRDRDDSLVCDCRHNTAGPECDRCKPFHYDRPWQRATAREANECVACNCNLHARRCRFNMELYKLSGRKSGGVCLNCRHNTAGRHCHYCKEGYYRDMGKPITHRKACKACDCHPVGAAGKTCNQTTGQCPCKDGVTGITCNRCAKGYQQSRSPIAPCIKIPVAPPTTAASSVEEPEDCDSYCKASKGKLKINMKKYCKKDYAVQIHILKADKAGDWWKFTVNIISVYKQGTSRIRRGDQSLWIRSRDIACKCPKIKPLKKYLLLGNAEDSPDQSGIVADKSSLVIQWRDTWARRLRKFQQREKKGKCKKA

SEQ ID NO: 29 - DNA, 1503 bp, Homo sapiens
  source 1..1503: mol_type = other DNA
  CDS 1..1503
atgagcaactccgttcctctgctctgtttctggagcctctgctattgctttgctgcggggagccccgtaccttttggtccagagggacggctggaagataagctccacaaacccaaagctacacagactgaggtcaaaccatctgtgaggtttaacctccgcacctccaaggacccagagcatgaaggatgctacctctccgtcggccacagccagcccttagaagactgcagtttcaacatgacagctaaaacctttttcatcattcacggatggacgatgagcggtatctttgaaaactggctgcacaaactcgtgtcagccctgcacacaagagagaaagacgccaatgtagttgtggttgactggctccccctggcccaccagctttacacggatgcggtcaataataccagggtggtgggacacagcattgccaggatgctcgactggctgcaggagaaggacgatttttctctcgggaatgtccacttgatcggctacagcctcggagcgcacgtggccgggtatgcaggcaacttcgtgaaaggaacggtgggccgaatcacaggtttggatcctgccgggcccatgtttgaaggggccgacatccacaagaggctctctccggacgatgcagattttgtggatgtcctccacacctacacgcgttccttcggcttgagcattggtattcagatgcctgtgggccacattgacatctaccccaatgggggtgacttccagccaggctgtggactcaacgatgtcttgggatcaattgcatatggaacaatcacagaggtggtaaaatgtgagcatgagcgagccgtccacctctttgttgactctctggtgaatcaggacaagccgagttttgccttccagtgcactgactccaatcgcttcaaaaaggggatctgtctgagctgccgcaagaaccgttgtaatagcattggctacaatgccaagaaaatgaggaacaagaggaacagcaaaatgtacctaaaaacccgggcaggcatgcctttcagagtttaccattatcagatgaaaatccatgtcttcagttacaagaacatgggagaaattgagcccaccttttacgtcaccctttatggcactaatgcagattcccagactctgccactggaaatagtggagcggatcgagcagaatgccaccaacaccttcctggtctacaccgaggaggacttgggagacctcttgaagatccagctcacctgggagggggcctctcagtcttggtacaacctgtggaaggagtttcgcagctacctgtctcaaccccgcaaccccggacgggagctgaatatcaggcgcatccgggtgaagtctggggaaacccagcggaaactgacattttgtacagaagaccctgagaacaccagcatatccccaggccgggagctctggtttcgcaagtgtcgggatggctggaggatgaaaaacgaaaccagtcccactgtggagcttccctga

SEQ ID NO: 30 - protein, 500 aa, Homo sapiens
MSNSVPLLCFWSLCYCFAAGSPVPFGPEGRLEDKLHKPKATQTEVKPSVRFNLRTSKDPEHEGCYLSVGHSQPLEDCSFNMTAKTFFIIHGWTMSGIFENWLHKLVSALHTREKDANVVVVDWLPLAHQLYTDAVNNTRVVGHSIARMLDWLQEKDDFSLGNVHLIGYSLGAHVAGYAGNFVKGTVGRITGLDPAGPMFEGADIHKRLSPDDADFVDVLHTYTRSFGLSIGIQMPVGHIDIYPNGGDFQPGCGLNDVLGSIAYGTITEVVKCEHERAVHLFVDSLVNQDKPSFAFQCTDSNRFKKGICLSCRKNRCNSIGYNAKKMRNKRNSKMYLKTRAGMPFRVYHYQMKIHVFSYKNMGEIEPTFYVTLYGTNADSQTLPLEIVERIEQNATNTFLVYTEEDLGDLLKIQLTWEGASQSWYNLWKEFRSYLSQPRNPGRELNIRRIRVKSGETQRKLTFCTEDPENTSISPGRELWFRKCRDGWRMKNETSPTVELP

SEQ ID NO: 31 - DNA, 21 bp, synthetic construct
  misc_feature 1..21: note = Forward primer for amplification of HBV pregenome RNA
  source 1..21: mol_type = other DNA
gctctgtatcgggaggcctta

SEQ ID NO: 32 - DNA, 23 bp, synthetic construct
  misc_feature 1..23: note = Reverse primer for amplification of HBV pregenome RNA
  source 1..23: mol_type = other DNA
tgagtgctgtatggtgaggagaa

SEQ ID NO: 33 - DNA, 15 bp, synthetic construct
  misc_feature 1..15: note = qRT-PCR probe for detection of HBV pregenome RNA
  source 1..15: mol_type = other DNA
agtctccggaacatt

SEQ ID NO: 34 - DNA, 25 bp, synthetic construct
  misc_feature 1..25: note = Forward primer for amplification of LIPG
  source 1..25: mol_type = other DNA
ttagaattcatgagcaactccgttc

SEQ ID NO: 35 - DNA, 47 bp, synthetic construct
  misc_feature 1..47: note = Reverse primer for amplification of LIPG
  source 1..47: mol_type = other DNA
aattctagatcatctgctcatctgttgttgtgggaagctccacagtg

SEQ ID NO: 36 - DNA, 86 bp, synthetic construct
  misc_feature 1..86: note = primer GSP6-GFP-F
  source 1..86: mol_type = other DNA
ggaagatctatttaggtgacactatagaacaacaacaacaacaaacaacaacaaaatgagtaaaggagaagaacttttcactggag

SEQ ID NO: 37 - DNA, 26 bp, synthetic construct
  misc_feature 1..26: note = primer GFP-R
  source 1..26: mol_type = other DNA
tttgtatagttcatccatgccatgtg

SEQ ID NO: 38 - DNA, 31 bp, synthetic construct
  misc_feature 1..31: note = primer Flag-His-F
  source 1..31: mol_type = other DNA
gactataaggacgacgacgacaagcaccatc

SEQ ID NO: 39 - DNA, 51 bp, synthetic construct
  misc_feature 1..51: note = primer Atail (R)
  source 1..51: mol_type = other DNA
tttttttttcttgtagtagaactgggtgctggtcgtaatcccgccaatgcc

SEQ ID NO: 40 - DNA, 83 bp, synthetic construct
  misc_feature 1..83: note = primer 16NNS-F
  misc_feature 17..18: note = N is A, T, C or G.
  misc_feature 19: note = S is G or C.
  misc_feature 20..21: note = N is A, T, C or G.
  misc_feature 22: note = S is G or C.
  misc_feature 23..24: note = N is A, T, C or G.
  misc_feature 25: note = S is G or C.
  misc_feature 26..27: note = N is A, T, C or G.
  misc_feature 28: note = S is G or C.
  misc_feature 29..30: note = N is A, T, C or G.
  misc_feature 31: note = S is G or C.
  misc_feature 32..33: note = N is A, T, C or G.
  misc_feature 34: note = S is G or C.
  misc_feature 35..36: note = N is A, T, C or G.
  misc_feature 37: note = S is G or C.
  misc_feature 38..39: note = N is A, T, C or G.
  misc_feature 40: note = S is G or C.
  misc_feature 41..42: note = N is A, T, C or G.
  misc_feature 43: note = S is G or C.
  misc_feature 44..45: note = N is A, T, C or G.
  misc_feature 46: note = S is G or C.
  misc_feature 47..48: note = N is A, T, C or G.
  misc_feature 49: note = S is G or C.
  misc_feature 50..51: note = N is A, T, C or G.
  misc_feature 52: note = S is G or C.
  misc_feature 53..54: note = N is A, T, C or G.
  misc_feature 55: note = S is G or C.
  misc_feature 56..57: note = N is A, T, C or G.
  misc_feature 58: note = S is G or C.
  misc_feature 59..60: note = N is A, T, C or G.
  misc_feature 61: note = S is G or C.
  misc_feature 62..63: note = N is A, T, C or G.
  misc_feature 64: note = S is G or C.
  source 1..83: mol_type = other DNA
ggatgaactatacaaannsnnsnnsnnsnnsnnsnnsnnsnnsnnsnnsnnsnnsnnsnnsnnsgactataaggacgacgacg

SEQ ID NO: 41 - DNA, 70 bp, synthetic construct
  misc_feature 1..70: note = primer 9NNS-F
  misc_feature 25..26: note = N is A, T, G or C.
  misc_feature 27: note = S is G or C.
  misc_feature 28..29: note = N is A, T, G or C.
  misc_feature 30: note = S is G or C.
  misc_feature 31..32: note = N is A, T, G or C.
  misc_feature 33: note = S is G or C.
  misc_feature 34..35: note = N is A, T, G or C.
  misc_feature 36: note = S is G or C.
  misc_feature 37..38: note = N is A, T, G or C.
  misc_feature 39: note = S is G or C.
  misc_feature 40..41: note = N is A, T, G or C.
  misc_feature 42: note = S is G or C.
  misc_feature 43..44: note = N is A, T, G or C.
  misc_feature 45: note = S is G or C.
  misc_feature 46..47: note = N is A, T, G or C.
  misc_feature 48: note = S is G or C.
  misc_feature 49..50: note = N is A, T, G or C.
  misc_feature 51: note = S is G or C.
  source 1..70: mol_type = other DNA
catggcatggatgaactatacaaannsnnsnnsnnsnnsnnsnnsnnsnnsgactataaggacgacgacg

SEQ ID NO: 42 - protein, 29 aa, Homo sapiens
RKNRCNSIGYNAKKMRNKRNSKMYLKTRA

SEQ ID NO: 43 - DNA, 35 bp, synthetic construct
  misc_feature 1..35: note = primer LIPG-ifpc-F
  source 1..35: mol_type = other DNA
cggactctagaggatgccaccatgagcaactccgt

SEQ ID NO: 44 - DNA, 30 bp, synthetic construct
  misc_feature 1..30: note = primer LIPG-ifbio-R
  source 1..30: mol_type = other DNA
cggggtgccggcgccgggaagctccacagt

SEQ ID NO: 45 - DNA, 20 bp, synthetic construct
  misc_feature 1..20: note = primer F-Bio
  source 1..20: mol_type = other DNA
ggcgccggcaccccggtgac

SEQ ID NO: 46 - DNA, 20 bp, synthetic construct
  misc_feature 1..20: note = primer R-Bio
  source 1..20: mol_type = other DNA
cgccagggtcatcagggtgt

SEQ ID NO: 47 - DNA, 68 bp, synthetic construct
  misc_feature 1..68: note = primer Bio-Flag-Histag A stop
  source 1..68: mol_type = other DNA
ctaatggtgatggtggtgatggtgcttgtcgtcgtcgtccttgtagtccgccagggtcatcagggtgt

SEQ ID NO: 48 - DNA, 48 bp, synthetic construct
  misc_feature 1..48: note = primer Flag-Histag A stop
  source 1..48: mol_type = other DNA
ctaatggtgatggtggtgatggtgcttgtcgtcgtcgtccttgtagtc

SEQ ID NO: 49 - DNA, 35 bp, synthetic construct
  misc_feature 1..35: note = primer LIPG-hb-ifpc-F1
  source 1..35: mol_type = other DNA
gaggatgccaccatgcgcaagaaccgttgtaatag

SEQ ID NO: 50 - DNA, 35 bp, synthetic construct
  misc_feature 1..35: note = primer LIPG-hb-if-R1
  source 1..35: mol_type = other DNA
acaacggttcttgcgtgcccgggtttttaggtaca

SEQ ID NO: 51 - DNA, 20 bp, synthetic construct
  misc_feature 1..20: note = primer LIPG-hb-F2
  source 1..20: mol_type = other DNA
cgcaagaaccgttgtaatag

SEQ ID NO: 52 - DNA, 35 bp, synthetic construct
  misc_feature 1..35: note = primer LIPG-hb-if-R2
  source 1..35: mol_type = other DNA
tgaaccgcctccacctgcccgggtttttaggtaca

SEQ ID NO: 53 - DNA, 60 bp, synthetic construct
  misc_feature 1..60: note = primer Linker
  source 1..60: mol_type = other DNA
ggtggaggcggttcaggcggaggtggctctggcggtggcggatccggaggtggtggcagc

SEQ ID NO: 54 - DNA, 20 bp, synthetic construct
  misc_feature 1..20: note = primer GSlinker-F1
  source 1..20: mol_type = other DNA
ggtggaggcggttcaggcgg

SEQ ID NO: 55 - DNA, 35 bp, synthetic construct
  misc_feature 1..35: note = primer GSlinker-ifbio-R1
  source 1..35: mol_type = other DNA
cggggtgccggcgccgctgccaccacctccggatc

SEQ ID NO: 56 - DNA, 23 bp, synthetic construct
  misc_feature 1..23: note = primer pcDNA-KATG-inv
  source 1..23: mol_type = other DNA
catggtggcatcctctagagtcc

SEQ ID NO: 57 - DNA, 31 bp, synthetic construct
  misc_feature 1..31: note = primer GFP-F in
  source 1..31: mol_type = other DNA
atgagtaaaggagaagaacttttcactggag

SEQ ID NO: 58 - DNA, 30 bp, synthetic construct
  misc_feature 1..30: note = primer His-Atail-R in
  source 1..30: mol_type = other DNA
accgatcacaaacggatggtgatggtggtg

SEQ ID NO: 59 - DNA, 30 bp, synthetic construct
  misc_feature 1..30: note = primer Atail-F iv
  source 1..30: mol_type = other DNA
ccgtttgtgatcggtgccggtgttctgggc

SEQ ID NO: 60 - DNA, 46 bp, synthetic construct
  misc_feature 1..46: note = primer 3.3KIgk-GFP-Riv
  source 1..46: mol_type = other DNA
ttctcctttactcatgtcaccagtggaacctggaacccagagcagc

SEQ ID NO: 61 - DNA, 20 bp, synthetic construct
  misc_feature 1..20: note = qPCR forward primer for detection of HBV DNA and cccDNA
  source 1..20: mol_type = other DNA
actcaccaacctcctgtcct

SEQ ID NO: 62 - DNA, 20 bp, synthetic construct
  misc_feature 1..20: note = qPCR reverse primer for detection of HBV DNA and cccDNA
  source 1..20: mol_type = other DNA
gacaaacgggcaacatacct

SEQ ID NO: 63 - DNA, 24 bp, synthetic construct
  misc_feature 1..24: note = qPCR probe for detection of HBV DNA and cccDNA
  source 1..24: mol_type = other DNA
tatcgctggatgtgtctgcggcgt

SEQ ID NO: 64 - DNA, 59 bp, synthetic construct
  misc_feature 1..59: note = shRNA for Netrin-1 knockdown
  source 1..59: mol_type = other DNA
ccgggactgcgattcctactgcaagctcgagcttgcagtaggaatcgcagtcttttttg

SEQ ID NO: 65 - protein, 119 aa, Hepatitis B virus
  SITE 78: note = misc_feature - Xaa can be any naturally occurring amino acid
MGGWSSKPRKGMGTNLSVPNPLGFFPDHQLDPAFKANSZNPDWDLNPHKDNWPDANKVGVGAFGPGFIPPHGGLLGWXPQAQGILTTVPAAPPPASTNRQSGRQPTPLSPPLRDTHPQA

SEQ ID NO: 66 - protein, 47 aa, synthetic construct
  REGION 1..47: note = preS1 peptide
GGWSSKPRKGMGTNLSVPNPLGFFPDHQLDPAFKANSZNPDWDLNPH

SEQ ID NO: 67 - DNA, 21 bp, synthetic construct
  misc_feature 1..21: note = Forward primer for detection of liver HBV DNA
  source 1..21: mol_type = other DNA
cacatcaggattcctaggacc

SEQ ID NO: 68 - DNA, 20 bp, synthetic construct
  misc_feature 1..20: note = Reverse primer for detection of liver HBV DNA
  source 1..20: mol_type = other DNA
aggttggtgagtgattggag

SEQ ID NO: 69 - DNA, 26 bp, synthetic construct
  misc_feature 1..26: note = Probe for detection of liver HBV DNA
  source 1..26: mol_type = other DNA
cagagtctagactcgtggtggacttc

SEQ ID NO: 70 - DNA, 19 bp, synthetic construct
  misc_feature 1..19: note = Forward primer for detection of liver HBV cccDNA
  source 1..19: mol_type = other DNA
ctccccgtctgtgccttct

SEQ ID NO: 71 - DNA, 18 bp, synthetic construct
  misc_feature 1..18: note = Reverse primer for detection of liver HBV cccDNA
  source 1..18: mol_type = other DNA
gccccaaagccacccaag

SEQ ID NO: 72 - DNA, 27 bp, synthetic construct
  misc_feature 1..27: note = Probe for detection of liver HBV cccDNA
  source 1..27: mol_type = other DNA
cgtcgcatggaraccaccgtgaacgcc

SEQ ID NO: 73 - DNA, 21 bp, synthetic construct
  misc_feature 1..21: note = LIPG shRNA target sequence
  source 1..21: mol_type = other DNA
ttacacggatgcggtcaataa

SEQ ID NO: 74 - protein, 8 aa, synthetic construct
  REGION 1..8: note = FLAG tag
DYKDDDDK

SEQ ID NO: 75 - protein, 8 aa, synthetic construct
  REGION 1..8: note = modified LIPH4-NTNBs
  SITE 2: note = MISC_FEATURE - Xaa is any amino acid other than Cys and Ala.
NXRHNTAG

SEQ ID NO: 76 - protein, 8 aa, synthetic construct
  REGION 1..8: note = modified LIPH4-23s
  SITE 3: note = MISC_FEATURE - Xaa is any amino acid other than Cys and Ala.
LNXRDNTR

SEQ ID NO: 77 - protein, 9 aa, synthetic construct
  source 1..9: note = LIPH4-LNTNBs
LNCRHNTAG

SEQ ID NO: 78 - protein, 16 aa, synthetic construct
  source 1..16: note = LIPH4-N4BP1a
SNCRINTFRTVPIEQK

SEQ ID NO: 79 - protein, 9 aa, synthetic construct
  source 1..9: note = LIPH4-N4BP1b
SNCRINTFR

SEQ ID NO: 80 - protein, 10 aa, synthetic construct
  source 1..10: note = LIPH4-N4BP1c
TSNCRINTFR

SEQ ID NO: 81 - DNA, 2691 bp, Homo sapiens
  source 1..2691: mol_type = other DNA
  CDS 1..2691: protein_id = 82; translation = MAARAVLDEFTAPAEKAELLEQSRGRIEGLFGVSLAVLGALGAEEPLPARIWLQLCGAQEAVHSAKEYIKGICEPELEERECYPKDMHCIFVGAESLFLKSLIQDTCADLCILDIGLLGIRGSAEAVVMARSHIQQFVKLFENKENLPSSQKESEVKREFKQFVEAHADNYTMDLLILPTSLKKELLTLTQGEENLFETGDDEVIEMRDSQQTEFTQNAATGLNISRDETVLQEEARNKAGTPVSELTKQMDTVLSSSPDVLFDPINGLTPDEEALSNERICQKRRFSDSEERHTKKQFSLENVQEGEILHDAKTLAGNVIADLSDSSADSENLSPDIKETTEEMEYNILVNFFKTMGYSQEIVEKVIKVYGPSTEPLLLLEEIEKENKRFQEDREFSAGTVYPETNKTKNKGVYSSTNELTTDSTPKKTQAHTQQNMVEKFSQLPFKVEAKPCTSNCRINTFRTVPIEQKHEVWGSNQNYICNTDPETDGLSPSVASPSPKEVNFVSRGASSHQPRVPLFPENGLHQQPEPLLPNNMKSACEKRLGCCSSPHSKPNCSTLSPPMPLPQLLPSVTDARSAGPSDHIDSSVTGVQRFRDTLKIPYKLELKNEPGRTDLKHIVIDGSNVAITHGLKKFFSCRGIAIAVEYFWKLGNRNITVFVPQWRTRRDPNVTEQHFLTQLQELGILSLTPARMVFGERIASHDDRFLLHLADKTGGIIVTNDNFREFVNESVSWREIITKRLLQYTFVGDIFMVPDDPLGRSGPRLEEFLQKEVCLRDMQPLLSALPNVGMFDPSFRVPGTQAASTSHQPPTRIQGAPSSHWLPQQPHFPLLPALPSLQQNLPMPAQRSSAETNELREALLKIFPDSEQRLKIDQILVAHPYMKDLNALSAMVLD
atggcggcccgggcggtgctggacgagttcactgcgccagctgagaaggcggagctgctggagcagagccgcggccgtatcgagggcctgtttggcgtgagcctagccgtgctcggcgcgctaggggctgaggagccgctgcccgcgcgcatctggctgcagctctgcggggcgcaggaggcggtgcacagcgccaaggaatatattaaaggaatctgtgaacctgaactagaagaaagagaatgttaccccaaggacatgcactgcatttttgttggggcagagagcctgtttctgaaaagcttgattcaggatacttgtgctgacctctgcattctggacattggccttcttggcatcagaggaagtgctgaggctgtggtcatggctaggagtcacattcaacaatttgtaaagctctttgaaaataaagagaacctacccagtagtcagaaagaatcagaggtgaaaagggaattcaaacaatttgttgaagcccatgcagacaattacacaatggatttgttgattttgcccacttccttgaaaaaagaacttttgacactcacacaaggtgaggagaatctctttgaaacaggagatgatgaggttattgaaatgagagattctcaacaaacagagtttacacagaatgctgccacagggctgaatatttctagagatgaaactgttttgcaggaagaggcaagaaataaagctgggactcctgtttctgagcttacaaaacaaatggacacagtcctttctagctcaccagatgtgctttttgatccaataaatggtctaaccccagatgaagaggcactttccaatgagagaatttgtcagaaaaggagattttctgattctgaagaaaggcatacgaagaagcagttttctttggaaaatgttcaggagggggagattttacacgatgctaagacattggctggaaatgtaatagctgacctatctgattcttctgctgattctgaaaatttaagtccagatataaaagaaactactgaggaaatggaatacaacatcctcgtaaacttttttaaaaccatgggctactcccaagaaattgttgaaaaggtcattaaggtgtatggaccatctactgaaccattattgctcttagaggaaattgaaaaagaaaataaaagattccaagaagacagagaattttcagctggtacagtgtatccagagaccaacaaaaccaaaaataaaggtgtttatagcagcacaaatgagcttacaactgattccactccaaagaaaacacaggctcacacacagcaaaatatggtagaaaaattttctcagttaccattcaaagtggaagctaaaccatgtacctcaaattgtagaattaatactttcagaacagtgccaatagaacagaaacatgaagtctggggttcaaaccagaactacatttgtaacacagaccctgaaactgatggcctttcaccttctgttgcctctccaagtcccaaagaagtcaattttgtttcaaggggagcttcaagtcaccagcccagagttccactttttcctgaaaatggtttacaccagcagccagaacccttgcttccaaataatatgaaatctgcctgtgaaaaacgtttaggatgttgtagttctcctcattctaagccaaattgctcaaccctttctccaccaatgccactgccccagctgttaccttcggttactgatgcaaggtcggcaggaccttctgatcatattgattcctcagttactggggttcaaaggtttcgagatactctaaaaataccctacaagctggaattaaaaaatgaaccagggagaacggatttgaaacacattgttatagatgggagcaatgttgcaattacccatggtctgaaaaagttcttttcttgtcgtggaattgcaattgcagttgaatatttttggaagcttggcaacagaaacatcactgtatttgtccctcagtggagaacaaggcgtgatcctaatgtcacagaacagcacttcttaacccagctccaggagctcggaatattatctttaactcctgcccggatggtctttggagaaagaattgcttctcatgatgacaggtttctactacacttagcggacaaaactggtggcataattgtgacaaatgataatttcagagaatttgtgaatgagtcagtctcttggagagaaattattacaaaaaggctgctgcagtacacgttcgtgggggacatatttatggttcccgatgatcctctgggaagaagtggacctcgattagaggagtttcttcagaaggaagtctgtcttagagatatgcagcccctactcagtgccctgccaaatgtgggcatgtttgaccccagcttcagagtccctggcacccaggcagccagcaccagccaccagcctccgacccggattcagggagccccttcaagccactggctccctcagcagccccacttcccactgctgccagccctccccagtctccagcagaacctgcccatgccagctcagagatcttctgcagaaaccaacgagctgagggaagcccttctgaagatcttccctgactcagagcaaagactgaaaatagaccagatcttggtggcccacccatacatgaaagatctaaatgcgctttctgccatggtgttggattga

SEQ ID NO: 82 - protein, 896 aa, Homo sapiens
MAARAVLDEFTAPAEKAELLEQSRGRIEGLFGVSLAVLGALGAEEPLPARIWLQLCGAQEAVHSAKEYIKGICEPELEERECYPKDMHCIFVGAESLFLKSLIQDTCADLCILDIGLLGIRGSAEAVVMARSHIQQFVKLFENKENLPSSQKESEVKREFKQFVEAHADNYTMDLLILPTSLKKELLTLTQGEENLFETGDDEVIEMRDSQQTEFTQNAATGLNISRDETVLQEEARNKAGTPVSELTKQMDTVLSSSPDVLFDPINGLTPDEEALSNERICQKRRFSDSEERHTKKQFSLENVQEGEILHDAKTLAGNVIADLSDSSADSENLSPDIKETTEEMEYNILVNFFKTMGYSQEIVEKVIKVYGPSTEPLLLLEEIEKENKRFQEDREFSAGTVYPETNKTKNKGVYSSTNELTTDSTPKKTQAHTQQNMVEKFSQLPFKVEAKPCTSNCRINTFRTVPIEQKHEVWGSNQNYICNTDPETDGLSPSVASPSPKEVNFVSRGASSHQPRVPLFPENGLHQQPEPLLPNNMKSACEKRLGCCSSPHSKPNCSTLSPPMPLPQLLPSVTDARSAGPSDHIDSSVTGVQRFRDTLKIPYKLELKNEPGRTDLKHIVIDGSNVAITHGLKKFFSCRGIAIAVEYFWKLGNRNITVFVPQWRTRRDPNVTEQHFLTQLQELGILSLTPARMVFGERIASHDDRFLLHLADKTGGIIVTNDNFREFVNESVSWREIITKRLLQYTFVGDIFMVPDDPLGRSGPRLEEFLQKEVCLRDMQPLLSALPNVGMFDPSFRVPGTQAASTSHQPPTRIQGAPSSHWLPQQPHFPLLPALPSLQQNLPMPAQRSSAETNELREALLKIFPDSEQRLKIDQILVAHPYMKDLNALSAMVLD

SEQ ID NO: 83 - protein, 6 aa, synthetic construct
  source 1..6: note = ASGR3-10M heavy chain CDR1
SSYWIE

SEQ ID NO: 84 - protein, 17 aa, synthetic construct
  source 1..17: note = ASGR3-10M heavy chain CDR2
EILPGSGSTNYNEKFKG

SEQ ID NO: 85 - protein, 9 aa, synthetic construct
  source 1..9: note = ASGR3-10M heavy chain CDR3
YGNYDAMDY

SEQ ID NO: 86 - protein, 12 aa, synthetic construct
  source 1..12: note = ASGR3-10M light chain CDR1
RASQSVSSSYLA

SEQ ID NO: 87 - protein, 7 aa, synthetic construct
  source 1..7: note = ASGR3-10M light chain CDR2
YASSRAT

SEQ ID NO: 88 - protein, 9 aa, synthetic construct
  source 1..9: note = ASGR3-10M light chain CDR3
QQSSSTPFT

SEQ ID NO: 89 - protein, 6 aa, synthetic construct
  source 1..6: note = ASGR3-39D heavy chain CDR1
SNYGMA

SEQ ID NO: 90 - protein, 17 aa, synthetic construct
  source 1..17: note = ASGR3-39D heavy chain CDR2
TISYDGSFTYYRDSVKG

SEQ ID NO: 91 - protein, 11 aa, synthetic construct
  source 1..11: note = ASGR3-39D heavy chain CDR3
KGRQADTEEDF

SEQ ID NO: 92 - protein, 15 aa, synthetic construct
  source 1..15: note = ASGR3-39D light chain CDR1
RASQSVSISSHDLMQ

SEQ ID NO: 93 - protein, 7 aa, synthetic construct
  source 1..7: note = ASGR3-39D light chain CDR2
DAFNLAS

SEQ ID NO: 94 - protein, 9 aa, synthetic construct
  source 1..9: note = ASGR3-39D light chain CDR3
QQSKDYPYT

SEQ ID NO: 95 - protein, 6 aa, synthetic construct
  source 1..6: note = ASGR4-70D heavy chain CDR1
SNYGMA

SEQ ID NO: 96 - protein, 17 aa, synthetic construct
  source 1..17: note = ASGR4-70D heavy chain CDR2
TISYDGSITYYRDSVKG

SEQ ID NO: 97 - protein, 10 aa, synthetic construct
  source 1..10: note = ASGR4-70D heavy chain CDR3
AHHRNTKSDF

SEQ ID NO: 98 - protein, 15 aa, synthetic construct
  source 1..15: note = ASGR4-70D light chain CDR1
RASQSVSISSHDLMQ

SEQ ID NO: 99 - protein, 7 aa, synthetic construct
  source 1..7: note = ASGR4-70D light chain CDR2
DAFNLAS

SEQ ID NO: 100 - protein, 9 aa, synthetic construct
  source 1..9: note = ASGR4-70D light chain CDR3
QQSKDDPYT

SEQ ID NO: 101 - protein, 6 aa, synthetic construct
  source 1..6: note = ASGR5-24M heavy chain CDR1
SSFGMH

SEQ ID NO: 102 - protein, 17 aa, synthetic construct
  source 1..17: note = ASGR5-24M heavy chain CDR2
YISSGSSTIYYANTVKG

SEQ ID NO: 103 - protein, 12 aa, synthetic construct
  source 1..12: note = ASGR5-24M heavy chain CDR3
LGPTVVATPFAY

SEQ ID NO: 104 - protein, 11 aa, synthetic construct
  source 1..11: note = ASGR5-24M light chain CDR1
KASQDVSTAVA

SEQ ID NO: 105 - protein, 7 aa, synthetic construct
  source 1..7: note = ASGR5-24M light chain CDR2
SASYRYS

SEQ ID NO: 106 - protein, 9 aa, synthetic construct
  source 1..9: note = ASGR5-24M light chain CDR3
QQYNNYPLT

SEQ ID NO: 107 - protein, 28 aa, synthetic construct
  source 1..28: note = S28 peptide
PFVIGAGVLGALGTGIGGITTSTQFYYK

SEQ ID NO: 108 - protein, 39 aa, synthetic construct
  source 1..39: note = S39 peptide
PFVIGAGVLGALGTGIGGITTSTQFYYKLSQELNGDMER

SEQ ID NO: 109 - DNA, 27 bp, synthetic construct
  source 1..27: mol_type = other DNA; note = base sequence encoding nuclear localization signal
  CDS 1..27: protein_id = 110; translation = PAAKRVKLD
cctgctgccaagagggtcaagttggac

SEQ ID NO: 110 - protein, 9 aa, synthetic construct
  source 1..9: note = nuclear localization signal
PAAKRVKLD

SEQ ID NO: 111 - protein, 4 aa, synthetic construct
  source 1..4: note = Furin cleavage sequence
RVRR

SEQ ID NO: 112 - protein, 15 aa, synthetic construct
  source 1..15: note = (GGGGS)3 linker
GGGGSGGGGSGGGGS

SEQ ID NO: 113 - DNA, 876 bp, Homo sapiens
  source 1..876: mol_type = other DNA
  CDS 1..876: protein_id = 114; translation = MTKEYQDLQHLDNEESDHHQLRKGPPPPQPLLQRLCSGPRLLLLSLGLSLLLLVVVCVIGSQNSQLQEELRGLRETFSNFTASTEAQVKGLSTQGGNVGRKMKSLESQLEKQQKDLSEDHSSLLLHVKQFVSDLRSLSCQMAALQGNGSERTCCPVNWVEHERSCYWFSRSGKAWADADNYCRLEDAHLVVVTSWEEQKFVQHHIGPVNTWMGLHDQNGPWKWVDGTDYETGFKNWRPEQPDDWYGHGLGGGEDCAHFTDDGRWNDDVCQRPYRWVCETELDKASQEPPLL
atgaccaaggagtatcaagaccttcagcatctggacaatgaggagagtgaccaccatcagctcagaaaagggccacctcctccccagcccctcctgcagcgtctctgctccggacctcgcctcctcctgctctccctgggcctcagcctcctgctgcttgtggttgtctgtgtgatcggatcccaaaactcccagctgcaggaggagctgcggggcctgagagagacgttcagcaacttcacagcgagcacggaggcccaggtcaagggcttgagcacccagggaggcaatgtgggaagaaagatgaagtcgctagagtcccagctggagaaacagcagaaggacctgagtgaagatcactccagcctgctgctccacgtgaagcagttcgtgtctgacctgcggagcctgagctgtcagatggcggcgctccagggcaatggctcagaaaggacctgctgcccggtcaactgggtggagcacgagcgcagctgctactggttctctcgctccgggaaggcctgggctgacgccgacaactactgccggctggaggacgcgcacctggtggtggtcacgtcctgggaggagcagaaatttgtccagcaccacataggccctgtgaacacctggatgggcctccacgaccaaaacgggccctggaagtgggtggacgggacggactacgagacgggcttcaagaactggaggccggagcagccggacgactggtacggccacgggctcggaggaggcgaggactgtgcccacttcaccgacgacggccgctggaacgacgacgtctgccagaggccctaccgctgggtctgcgagacagagctggacaaggccagccaggagccacctctcctttaa

SEQ ID NO: 114 - protein, 291 aa, Homo sapiens
MTKEYQDLQHLDNEESDHHQLRKGPPPPQPLLQRLCSGPRLLLLSLGLSLLLLVVVCVIGSQNSQLQEELRGLRETFSNFTASTEAQVKGLSTQGGNVGRKMKSLESQLEKQQKDLSEDHSSLLLHVKQFVSDLRSLSCQMAALQGNGSERTCCPVNWVEHERSCYWFSRSGKAWADADNYCRLEDAHLVVVTSWEEQKFVQHHIGPVNTWMGLHDQNGPWKWVDGTDYETGFKNWRPEQPDDWYGHGLGGGEDCAHFTDDGRWNDDVCQRPYRWVCETELDKASQEPPLL

SEQ ID NO: 115 - DNA, 936 bp, Homo sapiens
  source 1..936: mol_type = other DNA
  CDS 1..936: protein_id = 116; translation = MAKDFQDIQQLSSEENDHPFHQGEGPGTRRLNPRRGNPFLKGPPPAQPLAQRLCSMVCFSLLALSFNILLLVVICVTGSQSEGHRGAQLQAELRSLKEAFSNFSSSTLTEVQAISTHGGSVGDKITSLGAKLEKQQQDLKADHDALLFHLKHFPVDLRFVACQMELLHSNGSQRTCCPVNWVEHQGSCYWFSHSGKAWAEAEKYCQLENAHLVVINSWEEQKFIVQHTNPFNTWIGLTDSDGSWKWVDGTDYRHNYKNWAVTQPDNWHGHELGGSEDCVEVQPDGRWNDDFCLQVYRWVCEKRRNATGEVA
atggccaaggactttcaagatatccagcagctgagctcggaggaaaatgaccatcctttccatcaaggtgaggggccaggcactcgcaggctgaatcccaggagaggaaatccatttttgaaagggccacctcctgcccagcccctggcacagcgtctctgctccatggtctgcttcagtctgcttgccctgagcttcaacatcctgctgctggtggtcatctgtgtgactgggtcccaaagtgagggtcacaggggtgcacagctgcaagccgagctgcggagcctgaaggaagctttcagcaacttctcctcgagcaccctgacggaggtccaggcaatcagcacccacggaggcagcgtgggtgacaagatcacatccctaggagccaagctggagaaacagcagcaggacctgaaagcagatcacgatgccctgctcttccatctgaagcacttccccgtggacctgcgcttcgtggcctgccagatggagctcctccacagcaacggctcccaaaggacctgctgccccgtcaactgggtggagcaccaaggcagctgctactggttctctcactccgggaaggcctgggctgaggcggagaagtactgccagctggagaacgcacacctggtggtcatcaactcctgggaggagcagaaattcattgtacaacacacgaaccccttcaatacctggataggtctcacggacagtgatggctcttggaaatgggtggatggcacagactataggcacaactacaagaactgggctgtcactcagccagataattggcacgggcacgagctgggtggaagtgaagactgtgttgaagtccagccggatggccgctggaacgatgacttctgcctgcaggtgtaccgctgggtgtgtgagaaaaggcggaatgccaccggcgaggtggcctga

SEQ ID NO: 116 - protein, 311 aa, Homo sapiens
MAKDFQDIQQLSSEENDHPFHQGEGPGTRRLNPRRGNPFLKGPPPAQPLAQRLCSMVCFSLLALSFNILLLVVICVTGSQSEGHRGAQLQAELRSLKEAFSNFSSSTLTEVQAISTHGGSVGDKITSLGAKLEKQQQDLKADHDALLFHLKHFPVDLRFVACQMELLHSNGSQRTCCPVNWVEHQGSCYWFSHSGKAWAEAEKYCQLENAHLVVINSWEEQKFIVQHTNPFNTWIGLTDSDGSWKWVDGTDYRHNYKNWAVTQPDNWHGHELGGSEDCVEVQPDGRWNDDFCLQVYRWVCEKRRNATGEVA

SEQ ID NO: 117 - DNA, 35 bp, synthetic construct
  source 1..35: mol_type = other DNA; note = primer ASGR1-ex-if-F1
gacgacgacgacaagcaaaactcccagctgcagga

SEQ ID NO: 118 - DNA, 35 bp, synthetic construct
  source 1..35: mol_type = other DNA; note = primer ASGR2-ex-if-F1
gacgacgacgacaagcaaagtgagggtcacagggg

SEQ ID NO: 119 - DNA, 35 bp, synthetic construct
  source 1..35: mol_type = other DNA; note = primer ASGR1-if-R2
ctaaccggtagggatttaaaggagaggtggctcct

SEQ ID NO: 120 - DNA, 35 bp, synthetic construct
  source 1..35: mol_type = other DNA; note = primer ASGR2-if-R2
ctaaccggtagggattcaggccacctcgccggtgg

SEQ ID NO: 121 - DNA, 46 bp, synthetic construct
  source 1..46: mol_type = other DNA; note = primer Flag His tag A02
tttttttttatggtgatggtggtgatggtgcttgtcgtcgtcgtcc

SEQ ID NO: 122 - DNA, 79 bp, synthetic construct
  source 1..79: mol_type = other DNA; note = primer SP6 Omega
atttaggtgacactatagaacaacaacaacaacaaacaacaacaaaatggctagcatgactggtggacagcaaatgggt

SEQ ID NO: 123 - DNA, 33 bp, synthetic construct
  source 1..33: mol_type = other DNA; note = primer T7-long-F
atggctagcatgactggtggacagcaaatgggt

SEQ ID NO: 124 - DNA, 37 bp, synthetic construct
  source 1..37: mol_type = other DNA; note = primer Flag(Histag) in R
atggtgatggtggtgatggtgcttgtcgtcgtcgtcc

SEQ ID NO: 125 - DNA, 30 bp, synthetic construct
  source 1..30: mol_type = other DNA; note = primer His-stop-topo F
caccaccatcaccattagaagggttcgatc

SEQ ID NO: 126 - DNA, 30 bp, synthetic construct
  source 1..30: mol_type = other DNA; note = primer Igk-T7-R
agtcatgctagccatgtcaccagtggaacc

SEQ ID NO: 127 - protein, 72 aa, synthetic construct
  source 1..72: note = cleavage sequence + LIPH4-23 + Flag-tag + His-tag + S28 + nuclear localization signal
RVRRLNCRDNTRPVMSAMTCDYKDDDDKHHHHHHHPFVIGAGVLGALGTGIGGITTSTQFYYKPAAKRVKLD

SEQ ID NO: 128 - protein, 64 aa, synthetic construct
  source 1..64: note = cleavage sequence + LIPH4-23S + Flag-tag + His-tag + S28 + nuclear localization signal
RVRRLNCRDNTRDYKDDDDKHHHHHHHPFVIGAGVLGALGTGIGGITTSTQFYYKPAAKRVKLD

SEQ ID NO: 129 - protein, 75 aa, synthetic construct
  source 1..75: note = cleavage sequence + LIPH4-23S + Flag-tag + His-tag + S39 + nuclear localization signal
RVRRLNCRDNTRDYKDDDDKHHHHHHHPFVIGAGVLGALGTGIGGITTSTQFYYKLSQELNGDMERPAAKRVKLD

SEQ ID NO: 130 - protein, 64 aa, synthetic construct
  source 1..64: note = cleavage sequence + LIPH4-NTNBs + Flag-tag + His-tag + S28 + nuclear localization signal
RVRRNCRHNTAGDYKDDDDKHHHHHHHPFVIGAGVLGALGTGIGGITTSTQFYYKPAAKRVKLD

SEQ ID NO: 131 - protein, 65 aa, synthetic construct
  source 1..65: note = cleavage sequence + LIPH4-NTNBs + Flag-tag + His-tag + S28 + nuclear localization signal
RVRRLNCRHNTAGDYKDDDDKHHHHHHHPFVIGAGVLGALGTGIGGITTSTQFYYKPAAKRVKLD

SEQ ID NO: 132 - protein, 76 aa, synthetic construct
  source 1..76: note = cleavage sequence + LIPH4-NTNBs + Flag-tag + His-tag + S39 + nuclear localization signal
RVRRLNCRHNTAGDYKDDDDKHHHHHHHPFVIGAGVLGALGTGIGGITTSTQFYYKLSQELNGDMERPAAKRVKLD

SEQ ID NO: 133 - protein, 72 aa, synthetic construct
  source 1..72: note = cleavage sequence + LIPH4-N4BP1a + Flag-tag + His-tag + S28 + nuclear localization signal
RVRRSNCRINTFRTVPIEQKDYKDDDDKHHHHHHHPFVIGAGVLGALGTGIGGITTSTQFYYKPAAKRVKLD

SEQ ID NO: 134 - protein, 65 aa, synthetic construct
  source 1..65: note = cleavage sequence + LIPH4-N4BP1b + Flag-tag + His-tag + S28 + nuclear localization signal
RVRRSNCRINTFRDYKDDDDKHHHHHHHPFVIGAGVLGALGTGIGGITTSTQFYYKPAAKRVKLD

SEQ ID NO: 135 - protein, 66 aa, synthetic construct
  source 1..66: note = cleavage sequence + LIPH4-N4BP1c + Flag-tag + His-tag + S28 + nuclear localization signal
RVRRTSNCRINTFRDYKDDDDKHHHHHHHPFVIGAGVLGALGTGIGGITTSTQFYYKPAAKRVKLD

SEQ ID NO: 136 - protein, 6 aa, synthetic construct
  UNSURE 4: note = D or H or I
NCRXNT

SEQ ID NO: 137 - DNA, 1281 bp, Homo sapiens
  source 1..1281: mol_type = other DNA
  CDS 1..1281: protein_id = 138; translation = MSNSVPLLCFWSLCYCFAAGSPVPFGPEGRLEDKLHKPKATQTEVKPSVRFNLRTSKDPEHEGCYLSVGHSQPLEDCSFNMTAKTFFIIHGWTMSGIFENWLHKLVSALHTREKDANVVVVDWLPLAHQLYTDAVNNTRVVGHSIARMLDWLQEKDDFSLGNVHLIGYSLGAHVAGYAGNFVKGTVGRITAITEVVKCEHERAVHLFVDSLVNQDKPSFAFQCTDSNRFKKGICLSCRKNRCNSIGYNAKKMRNKRNSKMYLKTRAGMPFRVYHYQMKIHVFSYKNMGEIEPTFYVTLYGTNADSQTLPLEIVERIEQNATNTFLVYTEEDLGDLLKIQLTWEGASQSWYNLWKEFRSYLSQPRNPGRELNIRRIRVKSGETQRKLTFCTEDPENTSISPGRELWFRKCRDGWRMKNETSPTVELP
atgagcaactccgttcctctgctctgtttctggagcctctgctattgctttgctgcggggagccccgtaccttttggtccagagggacggctggaagataagctccacaaacccaaagctacacagactgaggtcaaaccatctgtgaggtttaacctccgcacctccaaggacccagagcatgaaggatgctacctctccgtcggccacagccagcccttagaagactgcagtttcaacatgacagctaaaacctttttcatcattcacggatggacgatgagcggtatctttgaaaactggctgcacaaactcgtgtcagccctgcacacaagagagaaagacgccaatgtagttgtggttgactggctccccctggcccaccagctttacacggatgcggtcaataataccagggtggtgggacacagcattgccaggatgctcgactggctgcaggagaaggacgatttttctctcgggaatgtccacttgatcggctacagcctcggagcgcacgtggccgggtatgcaggcaacttcgtgaaaggaacggtgggccgaatcacagcaatcacagaggtggtaaaatgtgagcatgagcgagccgtccacctctttgttgactctctggtgaatcaggacaagccgagttttgccttccagtgcactgactccaatcgcttcaaaaaggggatctgtctgagctgccgcaagaaccgttgtaatagcattggctacaatgccaagaaaatgaggaacaagaggaacagcaaaatgtacctaaaaacccgggcaggcatgcctttcagagtttaccattatcagatgaaaatccatgtcttcagttacaagaacatgggagaaattgagcccaccttttacgtcaccctttatggcactaatgcagattcccagactctgccactggaaatagtggagcggatcgagcagaatgccaccaacaccttcctggtctacaccgaggaggacttgggagacctcttgaagatccagctcacctgggagggggcctctcagtcttggtacaacctgtggaaggagtttcgcagctacctgtctcaaccccgcaaccccggacgggagctgaatatcaggcgcatccgggtgaagtctggggaaacccagcggaaactgacattttgtacagaagaccctgagaacaccagcatatccccaggccgggagctctggtttcgcaagtgtcgggatggctggaggatgaaaaacgaaaccagtcccactgtggagcttccctga

SEQ ID NO: 138 - protein, 426 aa, Homo sapiens
MSNSVPLLCFWSLCYCFAAGSPVPFGPEGRLEDKLHKPKATQTEVKPSVRFNLRTSKDPEHEGCYLSVGHSQPLEDCSFNMTAKTFFIIHGWTMSGIFENWLHKLVSALHTREKDANVVVVDWLPLAHQLYTDAVNNTRVVGHSIARMLDWLQEKDDFSLGNVHLIGYSLGAHVAGYAGNFVKGTVGRITAITEVVKCEHERAVHLFVDSLVNQDKPSFAFQCTDSNRFKKGICLSCRKNRCNSIGYNAKKMRNKRNSKMYLKTRAGMPFRVYHYQMKIHVFSYKNMGEIEPTFYVTLYGTNADSQTLPLEIVERIEQNATNTFLVYTEEDLGDLLKIQLTWEGASQSWYNLWKEFRSYLSQPRNPGRELNIRRIRVKSGETQRKLTFCTEDPENTSISPGRELWFRKCRDGWRMKNETSPTVELP